European Patent Application EP 4 372 008 A2, published May 22, 2024. Title: TROPISM-MODIFIED RECOMBINANT VIRAL VECTORS AND USES THEREOF FOR THE TARGETED INTRODUCTION OF GENETIC MATERIAL INTO HUMAN CELLS. Applicant: Regeneron Pharmaceuticals, Inc. Application EP, filed June 27, 2018. The sequence listing filed with the application follows.

SEQUENCE LISTING (40 sequences)

SEQ ID NO: 1 - protein, 735 aa, adeno-associated virus 2 [sequence omitted]

SEQ ID NO: 2 - protein, 745 aa, synthetic construct
  REGION 1..745: note = AAV2 VP1 N587Myc
MAADGYLPDWLEDTLSEGIRQWWKLKPGPPPPKPAERHKDDSRGLVLPGYKYLGPFNGLDKGEPVNEADAAALEHDKAYDRQLDSGDNPYLKYNHADAEFQERLKEDTSFGGNLGRAVFQAKKRVLEPLGLVEEPVKTAPGKKRPVEHSPVEPDSSSGTGKAGQQPARKRLNFGQTGDADSVPDPQPLGQPPAAPSGLGTNTMATGSGAPMADNNEGADGVGNSSGNWHCDSTWMGDRVITTSTRTWALPTYNNHLYKQISSQSGASNDNHYFGYSTPWGYFDFNRFHCHFSPRDWQRLINNNWGFRPKRLNFKLFNIQVKEVTQNDGTTTIANNLTSTVQVFTDSEYQLPYVLGSAHQGCLPPFPADVFMVPQYGYLTLNNGSQAVGRSSFYCLEYFPSQMLRTGNNFTFSYTFEDVPFHSSYAHSQSLDRLMNPLIDQYLYYLSRTNTPSGTTTQSRLQFSQAGASDIRDQSRNWLPGPCYRQQRVSKTSADNNNSEYSWTGATKYHLNGRDSLVNPGPAMASHKDDEEKFFPQSGVLIFGKQGSEKTNVDIEKVMITDEEEIRTTNPVATEQYGSVSTNLQRGNEQKLISEEDLRQAATADVNTQGVLPGMVWQDRDVYLQGPIWAKIPHTDGHFHPSPLMGGFGLKHPPPQILIKNTPVPANPSTTFSAAKFASFITQYSTGQVSVEIEWELQKENSKRWNPEIQYTSNYNKSVNVDFTVDTNGVYSEPRPIGTRYLTRNL

SEQ ID NO: 3 - protein, 736 aa, adeno-associated virus 6
MAADGYLPDWLEDNLSEGIREWWDLKPGAPKPKANQQKQDDGRGLVLPGYKYLGPFNGLDKGEPVNAADAAALEHDKAYDQQLKAGDNPYLRYNHADAEFQERLQEDTSFGGNLGRAVFQAKKRVLEPFGLVEEGAKTAPGKKRPVEQSPQEPDSSSGIGKTGQQPAKKRLNFGQTGDSESVPDPQPLGEPPATPAAVGPTTMASGGGAPMADNNEGADGVGNASGNWHCDSTWLGDRVITTSTRTWALPTYNNHLYKQISSASTGASNDNHYFGYSTPWGYFDFNRFHCHFSPRDWQRLINNNWGFRPKRLNFKLFNIQVKEVTTNDGVTTIANNLTSTVQVFSDSEYQLPYVLGSAHQGCLPPFPADVFMIPQYGYLTLNNGSQAVGRSSFYCLEYFPSQMLRTGNNFTFSYTFEDVPFHSSYAHSQSLDRLMNPLIDQYLYYLNRTQNQSGSAQNKDLLFSRGSPAGMSVQPKNWLPGPCYRQQRVSKTKTDNNNSNFTWTGASKYNLNGRESIINPGTAMASHKDDKDKFFPMSGVMIFGKESAGASNTALDNVMITDEEEIKATNPVATERFGTVAVNLQSSSTDPATGDVHVMGALPGMVWQDRDVYLQGPIWAKIPHTDGHFHPSPLMGGFGLKHPPPQILIKNTPVPANPPAEFSATKFASFITQYSTGQVSVEIEWELQKENSKRWNPEVQYTSNYAKSANVDFTVDNNGLYTEPRPIGTRYLTRPL

SEQ ID NO: 4 - protein, 746 aa, synthetic construct
  REGION 1..746: note = AAV6 VP1 Q585Myc
MAADGYLPDWLEDNLSEGIREWWDLKPGAPKPKANQQKQDDGRGLVLPGYKYLGPFNGLDKGEPVNAADAAALEHDKAYDQQLKAGDNPYLRYNHADAEFQERLQEDTSFGGNLGRAVFQAKKRVLEPFGLVEEGAKTAPGKKRPVEQSPQEPDSSSGIGKTGQQPAKKRLNFGQTGDSESVPDPQPLGEPPATPAAVGPTTMASGGGAPMADNNEGADGVGNASGNWHCDSTWLGDRVITTSTRTWALPTYNNHLYKQISSASTGASNDNHYFGYSTPWGYFDFNRFHCHFSPRDWQRLINNNWGFRPKRLNFKLFNIQVKEVTTNDGVTTIANNLTSTVQVFSDSEYQLPYVLGSAHQGCLPPFPADVFMIPQYGYLTLNNGSQAVGRSSFYCLEYFPSQMLRTGNNFTFSYTFEDVPFHSSYAHSQSLDRLMNPLIDQYLYYLNRTQNQSGSAQNKDLLFSRGSPAGMSVQPKNWLPGPCYRQQRVSKTKTDNNNSNFTWTGASKYNLNGRESIINPGTAMASHKDDKDKFFPMSGVMIFGKESAGASNTALDNVMITDEEEIKATNPVATERFGTVAVNLQEQKLISEEDLSSSTDPATGDVHVMGALPGMVWQDRDVYLQGPIWAKIPHTDGHFHPSPLMGGFGLKHPPPQILIKNTPVPANPPAEFSATKFASFITQYSTGQVSVEIEWELQKENSKRWNPEVQYTSNYAKSANVDFTVDNNGLYTEPRPIGTRYLTRPL

SEQ ID NO: 5 - protein, 736 aa, adeno-associated virus 9
MAADGYLPDWLEDNLSEGIREWWALKPGAPQPKANQQHQDNARGLVLPGYKYLGPGNGLDKGEPVNAADAAALEHDKAYDQQLKAGDNPYLKYNHADAEFQERLKEDTSFGGNLGRAVFQAKKRLLEPLGLVEEAAKTAPGKKRPVEQSPQEPDSSAGIGKSGAQPAKKRLNFGQTGDTESVPDPQPIGEPPAAPSGVGSLTMASGGGAPVADNNEGADGVGSSSGNWHCDSQWLGDRVITTSTRTWALPTYNNHLYKQISNSTSGGSSNDNAYFGYSTPWGYFDFNRFHCHFSPRDWQRLINNNWGFRPKRLNFKLFNIQVKEVTDNNGVKTIANNLTSTVQVFTDSDYQLPYVLGSAHEGCLPPFPADVFMIPQYGYLTLNDGSQAVGRSSFYCLEYFPSQMLRTGNNFQFSYEFENVPFHSSYAHSQSLDRLMNPLIDQYLYYLSKTINGSGQNQQTLKFSVAGPSNMAVQGRNYIPGPSYRQQRVSTTVTQNNNSEFAWPGASSWALNGRNSLMNPGPAMASHKEGEDRFFPLSGSLIFGKQGTGRDNVDADKVMITNEEEIKTTNPVATESYGQVATNHQSAQAQAQTGWVQNQGILPGMVWQDRDVYLQGPIWAKIPHTDGNFHPSPLMGGFGMKHPPPQILIKNTPVPADPPTAFNKDKLNSFITQYSTGQVSVEIEWELQKENSKRWNPEIQYTSNYYKSNNVEFAVNTEGVYSEPRPIGTRYLTRNL

SEQ ID NO: 6 - protein, 10 aa, synthetic construct
  REGION 1..10: note = c-myc
EQKLISEEDL

SEQ ID NO: 7 - protein, 8 aa, synthetic construct
  REGION 1..8: note = FLAG
DYKDDDDK

SEQ ID NO: 8 - protein, 9 aa, synthetic construct
  REGION 1..9: note = HA
YPYDVPDYA

SEQ ID NO: 9 - DNA, 21 bp, synthetic construct
  misc_feature 1..21: note = Fwd ITR primer
  source 1..21: mol_type = other DNA
ggaacccctagtgatggagtt

SEQ ID NO: 10 - DNA, 16 bp, synthetic construct
  misc_feature 1..16: note = Rvs ITR primer
  source 1..16: mol_type = other DNA
cggcctcagtgagcga

SEQ ID NO: 11 - DNA, 21 bp, synthetic construct
  misc_feature 1..21: note = AAV2 ITRs probe
  source 1..21: mol_type = other DNA
cactccctctctgcgcgctcg

SEQ ID NO: 12 - DNA, 30 bp, synthetic construct
  misc_feature 1..30: note = c-myc
  source 1..30: mol_type = other DNA
gaacaaaaactcatctcagaagaggatctg

SEQ ID NO: 13 - DNA, 20 bp, synthetic construct
  misc_feature 1..20: note = pAAVRCBsiWF
  source 1..20: mol_type = other DNA
ggagtaccagctcccgtacg

SEQ ID NO: 14 - DNA, 43 bp, synthetic construct
  misc_feature 1..43: note = N587mycR
  source 1..43: mol_type = other DNA
ctcttctgagatgagtttttgttcgttgcctctctggaggttg

SEQ ID NO: 15 - DNA, 43 bp, synthetic construct
  misc_feature 1..43: note = N587mycF
  source 1..43: mol_type = other DNA
aaactcatctcagaagaggatctgagacaagcagctaccgcag

SEQ ID NO: 16 - DNA, 18 bp, synthetic construct
  misc_feature 1..18: note = pAAVRCPmeR
  source 1..18: mol_type = other DNA
tccgcccgctgtttaaac

SEQ ID NO: 17 - DNA, 24 bp, synthetic construct
  misc_feature 1..24: note = pAAVRC9BsiWF
  source 1..24: mol_type = other DNA
actcagactatcagctcccgtacg

SEQ ID NO: 18 - DNA, 41 bp, synthetic construct
  misc_feature 1..41: note = A589mycR
  source 1..41: mol_type = other DNA
ctcttctgagatgagtttttgttctgcttgggcactctggt

SEQ ID NO: 19 - DNA, 37 bp, synthetic construct
  misc_feature 1..37: note = A589mycF
  source 1..37: mol_type = other DNA
aaactcatctcagagaggatctgcaggcgcagaccgg

SEQ ID NO: 20 - DNA, 19 bp, synthetic construct
  misc_feature 1..19: note = pAAVRC9PmeR
  source 1..19: mol_type = other DNA
ctccgcccgctgtttaaac

SEQ ID NO: 21 - protein, 738 aa, adeno-associated virus 8
MAADGYLPDWLEDNLSEGIREWWALKPGAPKPKANQQKQDDGRGLVLPGYKYLGPFNGLDKGEPVNAADAAALEHDKAYDQQLQAGDNPYLRYNHADAEFQERLQEDTSFGGNLGRAVFQAKKRVLEPLGLVEEGAKTAPGKKRPVEPSPQRSPDSSTGIGKKGQQPARKRLNFGQTGDSESVPDPQPLGEPPAAPSGVGPNTMAAGGGAPMADNNEGADGVGSSSGNWHCDSTWLGDRVITTSTRTWALPTYNNHLYKQISNGTSGGATNDNTYFGYSTPWGYFDFNRFHCHFSPRDWQRLINNNWGFRPKRLSFKLFNIQVKEVTQNEGTKTIANNLTSTIQVFTDSEYQLPYVLGSAHQGCLPPFPADVFMIPQYGYLTLNNGSQAVGRSSFYCLEYFPSQMLRTGNNFQFTYTFEDVPFHSSYAHSQSLDRLMNPLIDQYLYYLSRTQTTGGTANTQTLGFSQGGPNTMANQAKNWLPGPCYRQQRVSTTTGQNNNSNFAWTAGTKYHLNGRNSLANPGIAMATHKDDEERFFPSNGILIFGKQNAARDNADYSDVMLTSEEEIKTTNPVATEEYGIVADNLQQQNTAPQIGTVNSQGALPGMVWQNRDVYLQGPIWAKIPHTDGNFHPSPLMGGFGLKHPPPQILIKNTPVPADPPTTFNQSKLNSFITQYSTGQVSVEIEWELQKENSKRWNPEIQYTSNYYKSTSVDFAVNTEGVYSEPRPIGTRYLTRNL

SEQ ID NO: 22 - DNA, 453 bp, synthetic construct
  misc_feature 1..453: note = AAV8 N590myc gblock
  source 1..453: mol_type = other DNA
gaccctgttaccgccaacaacgcgtctcaacgacaaccgggcaaaacaacaatagcaactttgcctggactgctgggaccaaataccatctgaatggaagaaattcattggctaatcctggcatcgctatggcaacacacaaagacgacgaggagcgtttttttcccagtaacgggatcctgatttttggcaaacaaaatgctgccagagacaatgcggattacagcgatgtcatgctcaccagcgaggaagaaatcaaaaccactaaccctgtggctacagaggaatacggtatcgtggcagataacttgcagcagcaaaacgaacaaaaactcatctcagaagaggatctgacggctcctcaaattggaactgtcaacagccagggggccttacccggtatggtctggcagaaccgggacgtgtacctgcagggtcccatctgggccaaga

SEQ ID NO: 23 - DNA, 7336 bp, synthetic construct
  misc_feature 1..7336: note = pAAV RC2/8
  source 1..7336: mol_type = other DNA
gcgcgccgatatcgttaacgccccgcgccggccgctctagaactagtggatcccccggaagatcagaagttcctattccgaagttcctattctctagaaagtataggaacttctgatctgcgcagccgccatgccggggttttacgagattgtgattaaggtccccagcgaccttgacgagcatctgcccggcatttctgacagctttgtgaactgggtggccgagaaggaatgggagttgccgccagattctgacatggatctgaatctgattgagcaggcacccctgaccgtggccgagaagctgcagcgcgactttctgacggaatggcgccgtgtgagtaaggccccggaggcccttttctttgtgcaatttgagaagggagagagctacttccacatgcacgtgctcgtggaaaccaccggggtgaaatccatggttttgggacgtttcctgagtcagattcgcgaaaaactgattcagagaatttaccgcgggatcgagccgactttgccaaactggttcgcggtcacaaagaccagaaatggcgccggaggcgggaacaaggtggtggatgagtgctacatccccaattacttgctccccaaaacccagcctgagctccagtgggcgtggactaatatggaacagtatttaagcgcctgtttgaatctcacggagcgtaaacggttggtggcgcagcatctgacgcacgtgtcgcagacgcaggagcagaacaaagagaatcagaatcccaattctgatgcgccggtgatcagatcaaaaacttcagccaggtacatggagctggtcgggtggctcgtggacaaggggattacctcggagaagcagtggatccaggaggaccaggcctcatacatctccttcaatgcggcctccaactcgcggtcccaaatcaaggctgccttggacaatgcgggaaagattatgagcctgactaaaaccgcccccgactacctggtgggccagcagcccgtggaggacatttccagcaatcggatttataaaattttggaactaaacgggtacgatccccaatatgcggcttccgtctttctgggatgggccacgaaaaagttcggcaagaggaacaccatctggctgtttgggcctgcaactaccgggaagaccaacatcgcggaggccatagcccacactgtgcccttctacgggtgcgtaaactggaccaatgagaactttcccttcaacgactgtgtcgacaagatggtgatctggtgggaggaggggaagatgaccgccaaggtcgtggagtcggccaaagccattctcggaggaagcaaggtgcgcgtggaccagaaatgcaagtcctcggcccagatagacccgactcccgtgatcgtcacctccaacaccaacatgtgcgccgtgattgacgggaactcaacgaccttcgaacaccagcagccgttgcaagaccggatgttcaaatttgaactcacccgccgtctggatcatgactttgggaaggtcaccaagcaggaagtcaaagactttttccggtgggcaaaggatcacgtggttgaggtggagcatgaattctacgtcaaaaagggtggagccaagaaaagacccgcccccagtgacgcagatataagtgagcccaaacgggtgcgcgagtcagttgcgcagccatcgacgtcagacgcggaagcttcgatcaactacgcagacaggtaccaaaacaaatgttctcgtcacgtgggcatgaatctgatgctgtttccctgcagacaatgcgagagaatgaatcagaattcaaatatctgcttcactcacggacagaaagactgtttagagtgctttcccgtgtcagaatctcaacccgtttctgtcgtcaaaaaggcgtatcagaaactgtgctacattcatcatatcatgggaaaggtgccagacgcttgcactgcctgcgatctggtcaatgtggatttggatgactgcatctttgaacaataaatgatttaaatcaggtatggctgccgatggttatcttccagattggctcgaggacaacctctctgagggcattcgcgagtggtgggcgctgaaacctggagccccgaagcccaaagccaaccagcaaaagcaggacgacggccggggtctggtgcttcctggctacaagtacctcggacccttcaacggactcgacaagggggagcccgtcaacgcggcggacgcagcggccctcgagcacgacaaggcctacgaccagcagctgcaggcgggtgacaatccgtacctgcggtataaccacgccgacgccgagtttcaggagcgtctgcaagaagatacgtcttttgggggcaacctcgggcgagcagtcttccaggccaagaagcgggttctcgaacctctcggtctggttgaggaaggcgctaagacggctcctggaaagaagagaccggtagagccatcaccccagcgttctccagactcctctacgggcatcggcaagaaaggccaacagcccgccagaaaaagactcaattttggtcagactggcgactcagagtcagttccagaccctcaacctctcggagaacctccagcagcgccctctggtgtgggacctaatacaatggctgcaggcggtggcgcaccaatggcagacaataacgaaggcgccgacggagtgggtagttcctcgggaaattggcattgcgattccacatggctgggcgacagagtcatcaccaccagcacccgaacctgggccctgcccacctacaacaaccacctctacaagcaaatctccaacgggacatcgggaggagccaccaacgacaacacctacttcggctacagcaccccctgggggtattttgactttaacagattccactgccacttttcaccacgtgactggcagcgactcatcaacaacaactggggattccggcccaagagactcagcttcaagctcttcaacatccaggtcaaggaggtcacgcagaatgaaggcaccaagaccatcgccaataacctcaccagcaccatccaggtgtttacggactcggagtaccagctgccgtacgttctcggctctgcccaccagggctgcctgcctccgttcccggcggacgtgttcatgattccccagtacggctacctaacactcaacaacggtagtcaggccgtgggacgctcctccttctactgcctggaatactttccttcgcagatgctgagaaccggcaacaacttccagtttacttacaccttcgaggacgtgcctttccacagcagctacgcccacagccagagcttggaccggctgatgaatcctctgattgaccagtacctgtactacttgtctcggactcaaacaacaggaggcacggcaaatacgcagactctgggcttcagccaaggtgggcctaatacaatggccaatcaggcaaagaactggctgccaggaccctgttaccgccaacaacgcgtctcaacgacaaccgggcaaaacaacaatagcaactttgcctggactgctgggaccaaataccatctgaatggaagaaattcattggctaatcctggcatcgctatggcaacacacaaagacgacgaggagcgtttttttcccagtaacgggatcctgatttttggcaaacaaaatgctgccagagacaatgcggattacagcgatgtcatgctcaccagcgaggaagaaatcaaaaccactaaccctgtggctacagaggaatacggtatcgtggcagataacttgcagcagcaaaacacggctcctcaaattggaactgtcaacagccagggggccttacccggtatggtctggcagaaccgggacgtgtacctgcagggtcccatctgggccaagattcctcacacggacggcaacttccacccgtctccgctgatgggcggctttggcctgaaacatcctccgcctcagatcctgatcaagaacacgcctgtacctgcggatcctccgaccaccttcaaccagtcaaagctgaactctttcatcacgcaatacagcaccggacaggtcagcgtggaaattgaatgggagctgcagaaggaaaacagcaagcgctggaaccccgagatccagtacacctccaactactacaaatctacaagtgtggactttgctgttaatacagaaggcgtgtactctgaaccccgccccattggcacccgttacctcacccgtaatctgtaattgcctgttaatcaataaaccgtttaattcgtttcagttgaactttggtctctgcgtatttctttcttatctagtttccatggctacgtagataagtagcatggcgggttaatcattaactacagcccgggcgtttaaacagcgggcggaggggtggagtcgtgacgtgaattacgtcatagggttagggaggtcctgtattagaggtcacgtgagtgttttgcgacattttgcgacaccatgtggtctcgctgggggggggggcccgagtgagcacgcagggtctccattttgaagcgggaggtttgaacgagcgctggcgcgctcactggccgtcgttttacaacgtcgtgactgggaaaaccctggcgttacccaacttaatcgccttgcagcacatccccctttcgccagctggcgtaatagcgaagaggcccgcaccgatcgcccttcccaacagttgcgcagcctgaatggcgaatggaaattgtaagcgttaatattttgttaaaattcgcgttaaatttttgttaaatcagctcatttttttaaccaataggccgaaatcggcaaaatcccttataaatcaaaagaatagaccgagatagggttgagtgttgttccagtttggaacaagagtccactattaagaacgtggactccaacgtcaaagggcgaaaaaccgtctatcagggcgatggcccactacgtgaaccatcaccctaatcaagttttttggggtcgaggtgccgtaaagcactaaatcggaaccctaaagggagcccccgatttagagcttgacggggaaagccggcgaacgtggcgagaaaggaagggaagaaagcgaaaggagcgggcgctagggcgctggcaagtgtagcggtcacgctgcgcgtaaccaccacacccgccgcgcttaatgcgccgctacagggcgcgtcaggtggcacttttcggggaaatgtgcgcggaacccctatttgtttatttttctaaatacattcaaatatgtatccgctcatgagacaataaccctgataaatgcttcaataatattgaaaaaggaagagtatgagtattcaacatttccgtgtcgcccttattcccttttttgcggcattttgccttcctgtttttgctcacccagaaacgctggtgaaagtaaaagatgctgaagatcagttgggtgcacgagtgggttacatcgaactggatctcaacagcggtaagatccttgagagttttcgccccgaagaacgttttccaatgatgagcacttttaaagttctgctatgtggcgcggtattatcccgtattgacgccgggcaagagcaactcggtcgccgcatacactattctcagaatgacttggttgagtactcaccagtcacagaaaagcatcttacggatggcatgacagtaagagaattatgcagtgctgccataaccatgagtgataacactgcggccaacttacttctgacaacgatcggaggaccgaaggagctaaccgcttttttgcacaacatgggggatcatgtaactcgccttgatcgttgggaaccggagctgaatgaagccataccaaacgacgagcgtgacaccacgatgcctgtagcaatggcaacaacgttgcgcaaactattaactggcgaactacttactctagcttcccggcaacaattaatagactggatggaggcggataaagttgcaggaccacttctgcgctcggcccttccggctggctggtttattgctgataaatctggagccggtgagcgtgggtctcgcggtatcattgcagcactggggccagatggtaagccctcccgtatcgtagttatctacacgacggggagtcaggcaactatggatgaacgaaatagacagatcgctgagataggtgcctcactgattaagcattggtaactgtcagaccaagtttactcatatatactttagattgatttaaaacttcatttttaatttaaaaggatctaggtgaagatcctttttgataatctcatgaccaaaatcccttaacgtgagttttcgttccactgagcgtcagaccccgtagaaaagatcaaaggatcttcttgagatcctttttttctgcgcgtaatctgctgcttgcaaacaaaaaaaccaccgctaccagcggtggtttgtttgccggatcaagagctaccaactctttttccgaaggtaactggcttcagcagagcgcagataccaaatactgttcttctagtgtagccgtagttaggccaccacttcaagaactctgtagcaccgcctacatacctcgctctgctaatcctgttaccagtggctgctgccagtggcgataagtcgtgtcttaccgggttggactcaagacgatagttaccggataaggcgcagcggtcgggctgaacggggggttcgtgcacacagcccagcttggagcgaacgacctacaccgaactgagatacctacagcgtgagctatgagaaagcgccacgcttcccgaagggagaaaggcggacaggtatccggtaagcggcagggtcggaacaggagagcgcacgagggagcttccagggggaaacgcctggtatctttatagtcctgtcgggtttcgccacctctgacttgagcgtcgatttttgtgatgctcgtcaggggggcggagcctatggaaaaacgccagcaacgcggcctttttacggttcctggccttttgctggccttttgctcacatgttctttcctgcgttatcccctgattctgtggataaccgtattaccgcctttgagtgagctgataccgctcgccgcagccgaacgaccgagcgcagcgagtcagtgagcgaggaagcggaagagcgcccaatacgcaaaccgcctctccccgcgcgttggccgattcattaatgcagctggcacgacaggtttcccgactggaaagcgggcagtgagcgcaacgcaattaatgtgagttagctcactcattaggcaccccaggctttacactttatgcttccggctcgtatgttgtgtggaattgtgagcggataacaatttcacacaggaaacagctatgaccatgattacgccaa

SEQ ID NO: 24 - DNA, 7366 bp, synthetic construct
  misc_feature 1..7366: note = paav RC2/8 myc plasmid
  source 1..7366: mol_type = other DNA
gcgcgccgatatcgttaacgccccgcgccggccgctctagaactagtggatcccccggaagatcagaagttcctattccgaagttcctattctctagaaagtataggaacttctgatctgcgcagccgccatgccggggttttacgagattgtgattaaggtccccagcgaccttgacgagcatctgcccggcatttctgacagctttgtgaactgggtggccgagaaggaatgggagttgccgccagattctgacatggatctgaatctgattgagcaggcacccctgaccgtggccgagaagctgcagcgcgactttctgacggaatggcgccgtgtgagtaaggccccggaggcccttttctttgtgcaatttgagaagggagagagctacttccacatgcacgtgctcgtggaaaccaccggggtgaaatccatggttttgggacgtttcctgagtcagattcgcgaaaaactgattcagagaatttaccgcgggatcgagccgactttgccaaactggttcgcggtcacaaagaccagaaatggcgccggaggcgggaacaaggtggtggatgagtgctacatccccaattacttgctccccaaaacccagcctgagctccagtgggcgtggactaatatggaacagtatttaagcgcctgtttgaatctcacggagcgtaaacggttggtggcgcagcatctgacgcacgtgtcgcagacgcaggagcagaacaaagagaatcagaatcccaattctgatgcgccggtgatcagatcaaaaacttcagccaggtacatggagctggtcgggtggctcgtggacaaggggattacctcggagaagcagtggatccaggaggaccaggcctcatacatctccttcaatgcggcctccaactcgcggtcccaaatcaaggctgccttggacaatgcgggaaagattatgagcctgactaaaaccgcccccgactacctggtgggccagcagcccgtggaggacatttccagcaatcggatttataaaattttggaactaaacgggtacgatccccaatatgcggcttccgtctttctgggatgggccacgaaaaagttcggcaagaggaacaccatctggctgtttgggcctgcaactaccgggaagaccaacatcgcggaggccatagcccacactgtgcccttctacgggtgcgtaaactggaccaatgagaactttcccttcaacgactgtgtcgacaagatggtgatctggtgggaggaggggaagatgaccgccaaggtcgtggagtcggccaaagccattctcggaggaagcaaggtgcgcgtggaccagaaatgcaagtcctcggcccagatagacccgactcccgtgatcgtcacctccaacaccaacatgtgcgccgtgattgacgggaactcaacgaccttcgaacaccagcagccgttgcaagaccggatgttcaaatttgaactcacccgccgtctggatcatgactttgggaaggtcaccaagcaggaagtcaaagactttttccggtgggcaaaggatcacgtggttgaggtggagcatgaattctacgtcaaaaagggtggagccaagaaaagacccgcccccagtgacgcagatataagtgagcccaaacgggtgcgcgagtcagttgcgcagccatcgacgtcagacgcggaagcttcgatcaactacgcagacaggtaccaaaacaaatgttctcgtcacgtgggcatgaatctgatgctgtttccctgcagacaatgcgagagaatgaatcagaattcaaatatctgcttcactcacggacagaaagactgtttagagtgctttcccgtgtcagaatctcaacccgtttctgtcgtcaaaaaggcgtatcagaaactgtgctacattcatcatatcatgggaaaggtgccagacgcttgcactgcctgcgatctggtcaatgtggatttggatgactgcatctttgaacaataaatgatttaaatcaggtatggctgccgatggttatcttccagattggctcgaggacaacctctctgagggcattcgcgagtggtgggcgctgaaacctggagccccgaagcccaaagccaaccagcaaaagcaggacgacggccggggtctggtgcttcctggctacaagtacctcggacccttcaacggactcgacaagggggagcccgtcaacgcggcggacgcagcggccctcgagcacgacaaggcctacgaccagcagctgcaggcgggtgacaatccgtacctgcggtataaccacgccgacgccgagtttcaggagcgtctgcaagaagatacgtcttttgggggcaacctcgggcgagcagtcttccaggccaagaagcgggttctcgaacctctcggtctggttgaggaaggcgctaagacggctcctggaaagaagagaccggtagagccatcaccccagcgttctccagactcctctacgggcatcggcaagaaaggccaacagcccgccagaaaaagactcaattttggtcagactggcgactcagagtcagttccagaccctcaacctctcggagaacctccagcagcgccctctggtgtgggacctaatacaatggctgcaggcggtggcgcaccaatggcagacaataacgaaggcgccgacggagtgggtagttcctcgggaaattggcattgcgattccacatggctgggcgacagagtcatcaccaccagcacccgaacctgggccctgcccacctacaacaaccacctctacaagcaaatctccaacgggacatcgggaggagccaccaacgacaacacctacttcggctacagcaccccctgggggtattttgactttaacagattccactgccacttttcaccacgtgactggcagcgactcatcaacaacaactggggattccggcccaagagactcagcttcaagctcttcaacatccaggtcaaggaggtcacgcagaatgaaggcaccaagaccatcgccaataacctcaccagcaccatccaggtgtttacggactcggagtaccagctgccgtacgttctcggctctgcccaccagggctgcctgcctccgttcccggcggacgtgttcatgattccccagtacggctacctaacactcaacaacggtagtcaggccgtgggacgctcctccttctactgcctggaatactttccttcgcagatgctgagaaccggcaacaacttccagtttacttacaccttcgaggacgtgcctttccacagcagctacgcccacagccagagcttggaccggctgatgaatcctctgattgaccagtacctgtactacttgtctcggactcaaacaacaggaggcacggcaaatacgcagactctgggcttcagccaaggtgggcctaatacaatggccaatcaggcaaagaactggctgccaggaccctgttaccgccaacaacgcgtctcaacgacaaccgggcaaaacaacaatagcaactttgcctggactgctgggaccaaataccatctgaatggaagaaattcattggctaatcctggcatcgctatggcaacacacaaagacgacgaggagcgtttttttcccagtaacgggatcctgatttttggcaaacaaaatgctgccagagacaatgcggattacagcgatgtcatgctcaccagcgaggaagaaatcaaaaccactaaccctgtggctacagaggaatacggtatcgtggcagataacttgcagcagcaaaacgaacaaaaactcatctcagaagaggatctgacggctcctcaaattggaactgtcaacagccagggggccttacccggtatggtctggcagaaccgggacgtgtacctgcagggtcccatctgggccaagattcctcacacggacggcaacttccacccgtctccgctgatgggcggctttggcctgaaacatcctccgcctcagatcctgatcaagaacacgcctgtacctgcggatcctccgaccaccttcaaccagtcaaagctgaactctttcatcacgcaatacagcaccggacaggtcagcgtggaaattgaatgggagctgcagaaggaaaacagcaagcgctggaaccccgagatccagtacacctccaactactacaaatctacaagtgtggactttgctgttaatacagaaggcgtgtactctgaaccccgccccattggcacccgttacctcacccgtaatctgtaattgcctgttaatcaataaaccgtttaattcgtttcagttgaactttggtctctgcgtatttctttcttatctagtttccatggctacgtagataagtagcatggcgggttaatcattaactacagcccgggcgtttaaacagcgggcggaggggtggagtcgtgacgtgaattacgtcatagggttagggaggtcctgtattagaggtcacgtgagtgttttgcgacattttgcgacaccatgtggtctcgctgggggggggggcccgagtgagcacgcagggtctccattttgaagcgggaggtttgaacgagcgctggcgcgctcactggccgtcgttttacaacgtcgtgactgggaaaaccctggcgttacccaacttaatcgccttgcagcacatccccctttcgccagctggcgtaatagcgaagaggcccgcaccgatcgcccttcccaacagttgcgcagcctgaatggcgaatggaaattgtaagcgttaatattttgttaaaattcgcgttaaatttttgttaaatcagctcatttttttaaccaataggccgaaatcggcaaaatcccttataaatcaaaagaatagaccgagatagggttgagtgttgttccagtttggaacaagagtccactattaagaacgtggactccaacgtcaaagggcgaaaaaccgtctatcagggcgatggcccactacgtgaaccatcaccctaatcaagttttttggggtcgaggtgccgtaaagcactaaatcggaaccctaaagggagcccccgatttagagcttgacggggaaagccggcgaacgtggcgagaaaggaagggaagaaagcgaaaggagcgggcgctagggcgctggcaagtgtagcggtcacgctgcgcgtaaccaccacacccgccgcgcttaatgcgccgctacagggcgcgtcaggtggcacttttcggggaaatgtgcgcggaacccctatttgtttatttttctaaatacattcaaatatgtatccgctcatgagacaataaccctgataaatgcttcaataatattgaaaaaggaagagtatgagtattcaacatttccgtgtcgcccttattcccttttttgcggcattttgccttcctgtttttgctcacccagaaacgctggtgaaagtaaaagatgctgaagatcagttgggtgcacgagtgggttacatcgaactggatctcaacagcggtaagatccttgagagttttcgccccgaagaacgttttccaatgatgagcacttttaaagttctgctatgtggcgcggtattatcccgtattgacgccgggcaagagcaactcggtcgccgcatacactattctcagaatgacttggttgagtactcaccagtcacagaaaagcatcttacggatggcatgacagtaagagaattatgcagtgctgccataaccatgagtgataacactgcggccaacttacttctgacaacgatcggaggaccgaaggagctaaccgcttttttgcacaacatgggggatcatgtaactcgccttgatcgttgggaaccggagctgaatgaagccataccaaacgacgagcgtgacaccacgatgcctgtagcaatggcaacaacgttgcgcaaactattaactggcgaactacttactctagcttcccggcaacaattaatagactggatggaggcggataaagttgcaggaccacttctgcgctcggcccttccggctggctggtttattgctgataaatctggagccggtgagcgtgggtctcgcggtatcattgcagcactggggccagatggtaagccctcccgtatcgtagttatctacacgacggggagtcaggcaactatggatgaacgaaatagacagatcgctgagataggtgcctcactgattaagcattggtaactgtcagaccaagtttactcatatatactttagattgatttaaaacttcatttttaatttaaaaggatctaggtgaagatcctttttgataatctcatgaccaaaatcccttaacgtgagttttcgttccactgagcgtcagaccccgtagaaaagatcaaaggatcttcttgagatcctttttttctgcgcgtaatctgctgcttgcaaacaaaaaaaccaccgctaccagcggtggtttgtttgccggatcaagagctaccaactctttttccgaaggtaactggcttcagcagagcgcagataccaaatactgttcttctagtgtagccgtagttaggccaccacttcaagaactctgtagcaccgcctacatacctcgctctgctaatcctgttaccagtggctgctgccagtggcgataagtcgtgtcttaccgggttggactcaagacgatagttaccggataaggcgcagcggtcgggctgaacggggggttcgtgcacacagcccagcttggagcgaacgacctacaccgaactgagatacctacagcgtgagctatgagaaagcgccacgcttcccgaagggagaaaggcggacaggtatccggtaagcggcagggtcggaacaggagagcgcacgagggagcttccagggggaaacgcctggtatctttatagtcctgtcgggtttcgccacctctgacttgagcgtcgatttttgtgatgctcgtcaggggggcggagcctatggaaaaacgccagcaacgcggcctttttacggttcctggccttttgctggccttttgctcacatgttctttcctgcgttatcccctgattctgtggataaccgtattaccgcctttgagtgagctgataccgctcgccgcagccgaacgaccgagcgcagcgagtcagtgagcgaggaagcggaagagcgcccaatacgcaaaccgcctctccccgcgcgttggccgattcattaatgcagctggcacgacaggtttcccgactggaaagcgggcagtgagcgcaacgcaattaatgtgagttagctcactcattaggcaccccaggctttacactttatgcttccggctcgtatgttgtgtggaattgtgagcggataacaatttcacacaggaaacagctatgaccatgattacgccaa

SEQ ID NO: 25 - protein, 748 aa, synthetic construct
  REGION 1..748: note = pAAV8N590myc
MAADGYLPDWLEDNLSEGIREWWALKPGAPKPKANQQKQDDGRGLVLPGYKYLGPFNGLDKGEPVNAADAAALEHDKAYDQQLQAGDNPYLRYNHADAEFQERLQEDTSFGGNLGRAVFQAKKRVLEPLGLVEEGAKTAPGKKRPVEPSPQRSPDSSTGIGKKGQQPARKRLNFGQTGDSESVPDPQPLGEPPAAPSGVGPNTMAAGGGAPMADNNEGADGVGSSSGNWHCDSTWLGDRVITTSTRTWALPTYNNHLYKQISNGTSGGATNDNTYFGYSTPWGYFDFNRFHCHFSPRDWQRLINNNWGFRPKRLSFKLFNIQVKEVTQNEGTKTIANNLTSTIQVFTDSEYQLPYVLGSAHQGCLPPFPADVFMIPQYGYLTLNNGSQAVGRSSFYCLEYFPSQMLRTGNNFQFTYTFEDVPFHSSYAHSQSLDRLMNPLIDQYLYYLSRTQTTGGTANTQTLGFSQGGPNTMANQAKNWLPGPCYRQQRVSTTTGQNNNSNFAWTAGTKYHLNGRNSLANPGIAMATHKDDEERFFPSNGILIFGKQNAARDNADYSDVMLTSEEEIKTTNPVATEEYGIVADNLQQQNEQKLISEEDLTAPQIGTVNSQGALPGMVWQNRDVYLQGPIWAKIPHTDGNFHPSPLMGGFGLKHPPPQILIKNTPVPADPPTTFNQSKLNSFITQYSTGQVSVEIEWELQKENSKRWNPEIQYTSNYYKSTSVDFAVNTEGVYSEPRPIGTRYLTRNL

SEQ ID NO: 26 - protein, 746 aa, synthetic construct
  REGION 1..746: note = pAAV9A589myc
MAADGYLPDWLEDNLSEGIREWWALKPGAPQPKANQQHQDNARGLVLPGYKYLGPGNGLDKGEPVNAADAAALEHDKAYDQQLKAGDNPYLKYNHADAEFQERLKEDTSFGGNLGRAVFQAKKRLLEPLGLVEEAAKTAPGKKRPVEQSPQEPDSSAGIGKSGAQPAKKRLNFGQTGDTESVPDPQPIGEPPAAPSGVGSLTMASGGGAPVADNNEGADGVGSSSGNWHCDSQWLGDRVITTSTRTWALPTYNNHLYKQISNSTSGGSSNDNAYFGYSTPWGYFDFNRFHCHFSPRDWQRLINNNWGFRPKRLNFKLFNIQVKEVTDNNGVKTIANNLTSTVQVFTDSDYQLPYVLGSAHEGCLPPFPADVFMIPQYGYLTLNDGSQAVGRSSFYCLEYFPSQMLRTGNNFQFSYEFENVPFHSSYAHSQSLDRLMNPLIDQYLYYLSKTINGSGQNQQTLKFSVAGPSNMAVQGRNYIPGPSYRQQRVSTTVTQNNNSEFAWPGASSWALNGRNSLMNPGPAMASHKEGEDRFFPLSGSLIFGKQGTGRDNVDADKVMITNEEEIKTTNPVATESYGQVATNHQSAQAEQKLISEEDLQAQTGWVQNQGILPGMVWQDRDVYLQGPIWAKIPHTDGNFHPSPLMGGFGMKHPPPQILIKNTPVPADPPTAFNKDKLNSFITQYSTGQVSVEIEWELQKENSKRWNPEIQYTSNYYKSNNVEFAVNTEGVYSEPRPIGTRYLTRNL

SEQ ID NO: 27 - protein, 746 aa, synthetic construct
  REGION 1..746: note = pAAV9G453myc
MAADGYLPDWLEDNLSEGIREWWALKPGAPQPKANQQHQDNARGLVLPGYKYLGPGNGLDKGEPVNAADAAALEHDKAYDQQLKAGDNPYLKYNHADAEFQERLKEDTSFGGNLGRAVFQAKKRLLEPLGLVEEAAKTAPGKKRPVEQSPQEPDSSAGIGKSGAQPAKKRLNFGQTGDTESVPDPQPIGEPPAAPSGVGSLTMASGGGAPVADNNEGADGVGSSSGNWHCDSQWLGDRVITTSTRTWALPTYNNHLYKQISNSTSGGSSNDNAYFGYSTPWGYFDFNRFHCHFSPRDWQRLINNNWGFRPKRLNFKLFNIQVKEVTDNNGVKTIANNLTSTVQVFTDSDYQLPYVLGSAHEGCLPPFPADVFMIPQYGYLTLNDGSQAVGRSSFYCLEYFPSQMLRTGNNFQFSYEFENVPFHSSYAHSQSLDRLMNPLIDQYLYYLSKTINGEQKLISEEDLSGQNQQTLKFSVAGPSNMAVQGRNYIPGPSYRQQRVSTTVTQNNNSEFAWPGASSWALNGRNSLMNPGPAMASHKEGEDRFFPLSGSLIFGKQGTGRDNVDADKVMITNEEEIKTTNPVATESYGQVATNHQSAQAQAQTGWVQNQGILPGMVWQDRDVYLQGPIWAKIPHTDGNFHPSPLMGGFGMKHPPPQILIKNTPVPADPPTAFNKDKLNSFITQYSTGQVSVEIEWELQKENSKRWNPEIQYTSNYYKSNNVEFAVNTEGVYSEPRPIGTRYLTRNL

SEQ ID NO: 28 - DNA, 814 bp, synthetic construct
  misc_feature 1..814: note = cmyc-scfv-gblock
  source 1..814: mol_type = other DNA
tctccctgtctctgggtaaaggcggaggtggatccggagggggcggatctgacatccagatgacccagtctccatcctccctgtctgcatctgtaggagacagagtcaccatcacttgccgggcaagtcagagcattagcagctatttaaattggtatcaacagaaaccagggaaagcccctaagctcctgatctatgctgtttccattttgcaaagtggggtcccatcaaggttcagtggcagtggatctgggacagatttcactctcaccatcaactctctgcaacctgaagattttgcaacttactcctgtcaacagacttacagtacccctccgatcaccttcggccaagggacacgactggagattaaaggagggggcggctcaggaggagggggtagtgggggaggcggctccgaggtgcagctggtggagtctgggggaggcttggtacagcctggagggtccctgagactctcctgtgtcacctctggatttcgttttagtagttatgaaatgaactgggtccgccaggctccagggaaggggctggaatggatttcatacattaacagaagtggttataccatatactacgcagcctctctgaagggccgattcaccatctccagagacaacgccaagaactcactgtatcttcaaatgaacagcctgagagacgaggacacggctatctattactgtgcgagagggagtatcgcccctcggggggagattcgacacatctttgactactggggccagggaaccctggtcaccgtctcctcatgatgagcggccgctaatcagcc

SEQ ID NO: 29 - protein, 120 aa, synthetic construct
  REGION 1..120: note = myc HCVR AA
EVQLVESGGGLVQPGGSLRLSCVTSGFRFSSYEMNWVRQAPGKGLEWISYINRSGYTIYYAASLKGRFTISRDNAKNSLYLQMNSLRDEDTAIYYCARGSIAPRGEIRHIFDYWGQGTLV

SEQ ID NO: 30 - protein, 108 aa, synthetic construct
  REGION 1..108: note = myc LCVR AA
DIQMTQSPSSLSASVGDRVTITCRASQSISSYLNWYQQKPGKAPKLLIYAASSLQSGVPSRFSGSGSGTDFTLTISSLQPEDFATYYCQQSYSTPPITFGQGTRLEIK

SEQ ID NO: 31 - protein, 8 aa, synthetic construct
  REGION 1..8: note = myc HCDR1
GFRFSSYE

SEQ ID NO: 32 - protein, 8 aa, synthetic construct
  REGION 1..8: note = myc HCDR2 AA
INRSGYTI

SEQ ID NO: 33 - skipped

SEQ ID NO: 34 - protein, 6 aa, synthetic construct
  REGION 1..6: note = myc LCDR1 AA
QSISSY

SEQ ID NO: 35 - skipped

SEQ ID NO: 36 - protein, 7 aa, synthetic construct
  REGION 1..7: note = myc LCDR3 AA
QQSYSTP

SEQ ID NO: 37 - protein, 247 aa, synthetic construct
  REGION 1..247: note = anti-myc scFv
DIQMTQSPSSLSASVGDRVTITCRASQSISSYLNWYQQKPGKAPKLLIYAVSILQSGVPSRFSGSGSGTDFTLTINSLQPEDFATYSCQQTYSTPPITFGQGTRLEIKGGGGSGGGGSGGGGSEVQLVESGGGLVQPGGSLRLSCVTSGFRFSSYEMNWVRQAPGKGLEWISYINRSGYTIYYAASLKGRFTISRDNAKNSLYLQMNSLRDEDTAIYYCARGSIAPRGEIRHIFDYWGQGTLVTVSS

SEQ ID NO: 38 - DNA, 774 bp, synthetic construct
  misc_feature 1..774: note = anti-myc scFv NA
  source 1..774: mol_type = other DNA
ggcggaggtggatccggagggggcggatctgacatccagatgacccagtctccatcctccctgtctgcatctgtaggagacagagtcaccatcacttgccgggcaagtcagagcattagcagctatttaaattggtatcaacagaaaccagggaaagcccctaagctcctgatctatgctgtttccattttgcaaagtggggtcccatcaaggttcagtggcagtggatctgggacagatttcactctcaccatcaactctctgcaacctgaagattttgcaacttactcctgtcaacagacttacagtacccctccgatcaccttcggccaagggacacgactggagattaaaggagggggcggctcaggaggagggggtagtgggggaggcggctccgaggtgcagctggtggagtctgggggaggcttggtacagcctggagggtccctgagactctcctgtgtcacctctggatttcgttttagtagttatgaaatgaactgggtccgccaggctccagggaaggggctggaatggatttcatacattaacagaagtggttataccatatactacgcagcctctctgaagggccgattcaccatctccagagacaacgccaagaactcactgtatcttcaaatgaacagcctgagagacgaggacacggctatctattactgtgcgagagggagtatcgcccctcggggggagattcgacacatctttgactactggggccagggaaccctggtcaccgtctcctcatga

SEQ ID NO: 39 - DNA, 372 bp, synthetic construct
  misc_feature 1..372: note = myc HCVR NA
  source 1..372: mol_type = other DNA
gaggtgcagctggtggagtctgggggaggcttggtacagcctggagggtccctgagactctcctgtgtcacctctggatttcgttttagtagttatgaaatgaactgggtccgccaggctccagggaaggggctggaatggatttcatacattaacagaagtggttataccatatactacgcagcctctctgaagggccgattcaccatctccagagacaacgccaagaactcactgtatcttcaaatgaacagcctgagagacgaggacacggctatctattactgtgcgagagggagtatcgcccctcggggggagattcgacacatctttgactactggggccagggaaccctggtcaccgtctcctca

SEQ ID NO: 40 - DNA, 324 bp, synthetic construct
  misc_feature 1..324: note = myc LCVR NA
  source 1..324: mol_type = other DNA
gacatccagatgacccagtctccatcctccctgtctgcatctgtaggagacagagtcaccatcacttgccgggcaagtcagagcattagcagctatttaaattggtatcagcagaaaccagggaaagcccctaagctcctgatctatgctgcatccagtttgcaaagtggggtcccgtcaaggttcagtggcagtggatctgggacagatttcactctcaccatcagcagtctgcaacctgaagattttgcaacttactactgtcaacagagttacagtacccctccgatcaccttcggccaagggacacgactggagattaaa